European Patent Specification EP 3 460 044 B1, published January 24, 2024. Title: RECOMBINANT POLYNUCLEOTIDE SEQUENCE FOR PRODUCING ASTAXANTHIN AND USES THEREOF. Applicant: Academia Sinica. The sequence listing filed with the application follows.

SEQUENCE LISTING (140 sequences)

SEQ ID NO: 1 - DNA, 1128 bp, Artificial Sequence
  crtE gene
atggactacgccaacatcctcaccgccatccccctcgagttcaccccccaggacgacatcgtcctcctcgagccctaccactacctcggcaagaaccccggcaaggagatccgctcccagctcatcgaggccttcaactactggctcgacgtcaagaaggaggacctcgaggtcatccagaacgtcgtcggcatgctccacaccgcctccctcctcatggacgacgtcgaggactcctccgtcctccgccgcggctcccccgtcgcccacctcatctacggcatcccccagaccatcaacaccgccaactacgtctacttcctcgcctaccaggagatcttcaagctccgccccacccccatccccatgcccgtcatccccccctcctccgcctccctccagtcctccgtctcctccgcctcctcctcctcctccgcctcctccgagaacggcggcacctccacccccaactcccagatccccttctccaaggacacctacctcgacaaggtcatcaccgacgagatgctctccctccaccgcggccagggcctcgagctcttctggcgcgactccctcacctgcccctccgaggaggagtacgtcaagatggtcctcggcaagaccggcggcctcttccgcatcgccgtccgcctcatgatggccaagtccgagtgcgacatcgacttcgtccagctcgtcaacctcatctccatctacttccagatccgcgacgactacatgaacctccagtcctccgagtacgcccacaacaagaacttcgccgaggacctcaccgagggcaagttctccttccccaccatccactccatccacgccaacccctcctcccgcctcgtcatcaacaccctccagaagaagtccacctcccccgagatcctccaccactgcgtcaactacatgcgcaccgagacccactccttcgagtacacccaggaggtcctcaacaccctctccggcgccctcgagcgcgagctcggccgcctccagggcgagttcgccgaggccaactccaagatcgacctcggcgacgtcgagtccgagggccgcaccggcaagaacgtcaagctcgaggccatcctcaagaagctcgccgacatccccctc

SEQ ID NO: 2 - DNA, 1638 bp, Artificial Sequence
  HMG1 gene
atggagctcaccgccaacgacatccagaagaagcgcgccgccaagctcgtccccaagccctactccaaccacaacgagaagcagtccccctcctcctccgcctccaacgagaccaaggtcgagaccatcaccgagcgcatgcccgtcgtcgcctccatccagcacgagatcgacaccgagtccgactccgacaacggcccctccgaggtccgccccgtcgaggagctcgtcgaggtcctcaagggcggcgacgtcaagtccctctccaaccgcgaggtcgtctccctcgtcgtcgccaacaagctccccctctacgccctcgagaagcagctcggcgacaccacccgcgccgtcgtcgtccgccgcaaggccctcgccatcctcgccgacgcccccgtcctcaccaccgagcgcctcccctacaagaactacgactacaaccgcgtcttcggcgcctgctgcgagaacgtcatcggctacatgcccctccccgtcggcgtcatcggccccctcatgatcgacggcgtctactaccacatccccatggccaccaccgagggctgcctcgtcgcctccgccatgcgcggctgcaaggccatcaactccggcggcggcgtcaccaccgtcctcaccaaggacggcatgacccgcggcccctgcgtccgcttcccctccctcaagcgcgccggcgcctgcaagatctggctcgactccgaggagggccagaacaagatcaagaaggccttcaactccacctcccgcttcgcccgcctccagcacgtccagaccgccctcgccggcgacctcctcttcatccgcttccgcaccaccaccggcgacgccatgggcatgaacatgatctccaagggcgtcgagttctccctccaccagatggtcgaggagtacggctggaaggacatggagatcgtctccgtctccggcaactactgcatggacaagaagcccgccgccatcaactggatcgagggccgcggcaagtccgtcgtcgccgaggccaacatccccggcgacgtcgtccgcaaggtcctcaagtccgacgtcaaggccctcgtcgacctcaacatctccaagaacctcatcggctccgccatggccggctccatcggcggcttcaacgcccacgcctccaacctcgtcaccgccgtctacctcgccctcggccaggaccccgcccagaacgtcgagtcctccaactgcatgaccctcatgaaggaggtcgacggcgacctccgcatctccgtctccatgccctccatcgaggtcggcaccatcggcggcggcaccatcctcgagccccagtccgccatgctcgacctcctcggcgtccgcggcccccaccccaccgagcccggcaagaacgcccgccagctcgccaagatcgtcgcctccgccgtcatggccggcgagctctccctctgctccgccctcgccgccggccacctcgtccagtcccacatggtccacaaccgcgccaagcagcccgtcgccaccggcgccggcgcccccgtctccggccccggccccgtctccacccccgccatggccaccaacggcaaggagctctccgccgagcagctcaagaccctcaaggagggctccgtcatctgcatcaagtcc

SEQ ID NO: 3 - DNA, 1746 bp, Artificial Sequence
  crtI gene
atgggcaaggagcaggaccaggacaagcccaccgccatcatcgtcggctgcggcatcggcggcatcgccaccgccgcccgcctcgccaaggagggcttccaggtcaccgtcttcgagaagaacgactactccggcggccgctgctccctcatcgagcgcgacggctaccgcttcgaccagggcccctccctcctcctcctccccgacctcttcaagcagaccttcgaggacctcggcgagaagatggaggactgggtcgacctcatcaagtgcgagcccaactacgtctgccacttccacgacgaggagaccttcaccctctccaccgacatggccctcctcaagcgcgaggtcgagcgcttcgagggcaaggacggcttcgaccgcttcctctccttcatccaggaggcccaccgccactacgagctcgccgtcgtccacgtcctccagaagaacttccccggcttcgccgccttcctccgcctccagttcatcggccagatcctcgccctccaccccttcgagtccatctggacccgcgtctgccgctacttcaagaccgaccgcctccgccgcgtcttctccttcgccgtcatgtacatgggccagtccccctactccgcccccggcacctactccctcctccagtacaccgagctcaccgagggcatctggtacccccgcggcggcttctggcaggtccccaacaccctcctccagatcgtcaagcgcaacaacccctccgccaagttcaacttcaacgcccccgtctcccaggtcctcctctcccccgccaaggaccgcgccaccggcgtccgcctcgagtccggcgaggagcaccacgccgacgtcgtcatcgtcaacgccgacctcgtctacgcctccgagcacctcatccccgacgacgcccgcaacaagatcggccagctcggcgaggtcaagcgctcctggtgggccgacctcgtcggcggcaagaagctcaagggctcctgctcctccctctccttctactggtccatggaccgcatcgtcgacggcctcggcggccacaacatcttcctcgccgaggacttcaagggctccttcgacaccatcttcgaggagctcggcctccccgccgacccctccttctacgtcaacgtcccctcccgcatcgacccctccgccgcccccgagggcaaggacgccatcgtcatcctcgtcccctgcggccacatcgacgcctccaacccccaggactacaacaagctcgtcgcccgcgcccgcaagttcgtcatccacaccctctccgccaagctcggcctccccgacttcgagaagatgatcgtcgccgagaaggtccacgacgccccctcctgggagaaggagttcaacctcaaggacggctccatcctcggcctcgcccacaacttcatgcaggtcctcggcttccgcccctccacccgccaccccaagtacgacaagctcttcttcgtcggcgcctccacccaccccggcaccggcgtccccatcgtcctcgccggcgccaagctcaccgccaaccaggtcctcgagtccttcgaccgctcccccgcccccgaccccaacatgtccctctccgtcccctacggcaagcccctcaagtccaacggcaccggcatcgactcccaggtccagctcaagttcatggacctcgagcgctgggtctacctcctcgtcctcctcatcggcgccgtcatcgcccgctccgtcggcgtcctcgccttc

SEQ ID NO: 4 - DNA, 2019 bp, Artificial Sequence
  crtYB gene
atgaccgccctcgcctactaccagatccacctcatctacaccctccccatcctcggcctcctcggcctcctcacctcccccatcctcaccaagttcgacatctacaagatctccatcctcgtcttcatcgccttctccgccaccaccccctgggactcctggatcatccgcaacggcgcctggacctacccctccgccgagtccggccagggcgtcttcggcaccttcctcgacgtcccctacgaggagtacgccttcttcgtcatccagaccgtcatcaccggcctcgtctacgtcctcgccacccgccacctcctcccctccctcgccctccccaagacccgctcctccgccctctccctcgccctcaaggccctcatccccctccccatcatctacctcttcaccgcccacccctccccctcccccgaccccctcgtcaccgaccactacttctacatgcgcgccctctccctcctcatcaccccccccaccatgctcctcgccgccctctccggcgagtacgccttcgactggaagtccggccgcgccaagtccaccatcgccgccatcatgatccccaccgtctacctcatctgggtcgactacgtcgccgtcggccaggactcctggtccatcaacgacgagaagatcgtcggctggcgcctcggcggcgtcctccccatcgaggaggccatgttcttcctcctcaccaacctcatgatcgtcctcggcctctccgcctgcgaccacacccaggccctctacctcctccacggccgcaccatctacggcaacaagaagatgccctcctccttccccctcatcaccccccccgtcctctccctcttcttctcctcccgcccctactcctcccagcccaagcgcgacctcgagctcgccgtcaagctcctcgagaagaagtcccgctccttcttcgtcgcctccgccggcttcccctccgaggtccgcgagcgcctcgtcggcctctacgccttctgccgcgtcaccgacgacctcatcgactcccccgaggtctcctccaacccccacgccaccatcgacatggtctccgacttcctcaccctcctcttcggcccccccctccacccctcccagcccgacaagatcctctcctcccccctcctccccccctcccacccctcccgccccaccggcatgtaccccctccccccccccccctccctctcccccgccgagctcgtccagttcctcaccgagcgcgtccccgtccagtaccacttcgccttccgcctcctcgccaagctccagggcctcatcccccgctaccccctcgacgagctcctccgcggctacaccaccgacctcatcttccccctctccaccgaggccgtccaggcccgcaagacccccatcgagaccaccgccgacctcctcgactacggcctctgcgtcgccggctccgtcgccgagctcctcgtctacgtctcctgggcctccgccccctcccaggtccccgccaccatcgaggagcgcgaggccgtcctcgtcgcctcccgcgagatgggcaccgccctccagctcgtcaacatcgcccgcgacatcaagggcgacgccaccgagggccgcttctacctccccctctccttcttcggcctccgcgacgagtccaagctcgccatccccaccgactggaccgagccccgcccccaggacttcgacaagctcctctccctctccccctcctccaccctcccctcctccaacgcctccgagtccttccgcttcgagtggaagacctactccctccccctcgtcgcctacgccgaggacctcgccaagcactcctacaagggcatcgaccgcctccccaccgaggtccaggccggcatgcgcgccgcctgcgcctcctacctcctcatcggccgcgagatcaaggtcgtctggaagggcgacgtcggcgagcgccgcaccgtcgccggctggcgccgcgtccgcaaggtcctctccgtcgtcatgtccggctgggagggccag

SEQ ID NO: 5 - DNA, 891 bp, Artificial Sequence
  CrChYb gene
atgatgctcgcctcccgccccgccgtcgccctcggcgcccgcgcccagccccaggtcctccgccccaccctcgtcccccgccccggcatggtctccaacctccgcctccagcccgtcaaggtcgccgaccccatcgtcgcctccgagacctcccaggtcatggaggccccccaggagaagaagctctccgagttcgagctcaagcgcctcgagcgcaagcagcagcgcgcccaggaggccgccacctacaagttctccgccatcgccgccaccgtcctcgtcctctccatcgccgtcgtcgccacctactaccgcttcgcctggcacttcgccgaggacggcgacctccccgtcgacgagatggccgccaccctcctcctcgtcttcggcggcatgttcggcatggagatgtacgcccgcttcgcccacaaggtcctctggcacgacttcgagcccggctgggccctccacaagtcccaccacgagccccgcaccggccccttcgagctcaacgacatctacgccgtcgccaacgccctccccgccatggccctctgcgcctacggcttcttcaccccccacgtcatcggcggcgtctgcttcggcgccggcctcggcatcaccctcttcggcatcgcctacatgttcttccacgacggcctcgtccaccgccgcttccccgtcggccccatcgccaacctcccctacatgaagcgcatcatggtcgcccaccagatccaccacaccaacaagttcggcggcgtccccttcggcatgttcctcggcgtccaggagctcgaggccgtccccggcggcaaggaggagctcgacaagctcatggccgacctcgaggcccgcgaggccgccgccgccaaggccgccggctcctcc

SEQ ID NO: 6 - DNA, 897 bp, Artificial Sequence
  CzChYb gene
atgcagaccgtcttccagccctcctccgtctggcacctccgcaaccgccacgtcctcggcgaccgcacctgcgtcccctgccgcacctccctctccacctgccgccacgccgtccgcctcgtccgcgccaacgtcgccgagacccaggccacccccaccacctcccagatgctcgaggaggtccacgacgagtcccacgccgcctccgcctcctcccagatcttcgagctcgccgtcaagacctccatcaagcgccagcagcgcaaccgccagcagctcacctaccagggctccgccatcgccgcctccctcggcgtcggcgccctcgccgtcgccgccacccactacaagttctcctaccacatgccctccgagtcccccttcccctggctcgacatggccggcaccctcgccctcgtcatcggcggcgtcttcggcatggagatgtgggcccgctacgcccacaaggccctctggcacgacttccagcccggctgggccctccacaagtcccaccacgagccccgcatcggccccttcgaggccaacgacatcttcgccgtcatcaacgccgtccccgccttctccctctgcctctacggcttcctcacccccaacctcgtcggctccctctgcttcggcgccggcctcggcatcaccctcttcggcatcatgtacatgttcatccacgacggcctcgtccacaagcgcttccccgtcggccccatcgcccagatgcccgccatgaagcgcgtcgccatcgcccacaagctccaccactccgagaagtacggcggcgtcccctggggcatgttcttcggcccccaggagctcgaggccatcggcgccggccccgagctcgaccgcctctgcgccgagctcgactccaagtcctcc

SEQ ID NO: 7 - DNA, 879 bp, Artificial Sequence
  HpChYb gene
atgctctccaagctccagtccatctccgtcaaggcccgccgcgtcgagctcgcccgcgacatcacccgccccaaggtctgcctccacgcccagcgctgctccctcgtccgcctccgcgtcgccgccccccagaccgaggaggccctcggcaccgtccaggccgccggcgccggcgacgagcactccgccgacgtcgccctccagcagctcgaccgcgccatcgccgagcgccgcgcccgccgcaagcgcgagcagctctcctaccaggccgccgccatcgccgcctccatcggcgtctccggcatcgccatcttcgccacctacctccgcttcgccatgcacatgaccgtcggcggcgccgtcccctggggcgaggtcgccggcaccctcctcctcgtcgtcggcggcgccctcggcatggagatgtacgcccgctacgcccacaaggccatctggcacgagtcccccctcggctggctcctccacaagtcccaccacaccccccgcaccggccccttcgaggccaacgacctcttcgccatcatcaacggcctccccgccatgctcctctgcaccttcggcttctggctccccaacgtcctcggcgccgcctgcttcggcgccggcctcggcatcaccctctacggcatggcctacatgttcgtccacgacggcctcgtccaccgccgcttccccaccggccccatcgccggcctcccctacatgaagcgcctcaccgtcgcccaccagctccaccactccggcaagtacggcggcgccccctggggcatgttcctcggcccccaggagctccagcacatccccggcgccgccgaggaggtcgagcgcctcgtcctcgagctcgactggtccaagcgc

SEQ ID NO: 8 - DNA, 1332 bp, Artificial Sequence
  bkt gene
atgggccccggcatccagcccacctccgcccgcccctgctcccgcaccaagcactcccgcttcgccctcctcgccgccgccctcaccgcccgccgcgtcaagcagttcaccaagcagttccgctcccgccgcatggccgaggacatcctcaagctctggcagcgccagtaccacctcccccgcgaggactccgacaagcgcaccctccgcgagcgcgtccacctctaccgccccccccgctccgacctcggcggcatcgccgtcgccgtcaccgtcatcgccctctgggccaccctcttcgtctacggcctctggttcgtcaagctcccctgggccctcaaggtcggcgagaccgccacctcctgggccaccatcgccgccgtcttcttctccctcgagttcctctacaccggcctcttcatcaccacccacgacgccatgcacggcaccatcgccctccgcaaccgccgcctcaacgacttcctcggccagctcgccatctccctctacgcctggttcgactactccgtcctccaccgcaagcactgggagcaccacaaccacaccggcgagccccgcgtcgaccccgacttccaccgcggcaaccccaacctcgccgtctggttcgcccagttcatggtctcctacatgaccctctcccagttcctcaagatcgccgtctggtccaacctcctcctcctcgccggcgcccccctcgccaaccagctcctcttcatgaccgccgcccccatcctctccgccttccgcctcttctactacggcacctacgtcccccaccaccccgagaagggccacaccggcgccatgccctggcaggtctcccgcacctcctccgcctcccgcctccagtccttcctcacctgctaccacttcgacctccactgggagcaccaccgctggccctacgccccctggtgggagctccccaagtgccgccagatcgcccgcggcgccgccctcgcccccggccccctccccgtccccgccgccgccgccgccaccgccgccaccgccgccgccgccgccgccgccaccggctcccccgcccccgcctcccgcgccggctccgcctcctccgcctccgccgccgcctccggcttcggctccggccactccggctccgtcgccgcccagcccctctcctccctccccctcctctccgagggcgtcaagggcctcgtcgagggcgccatggagctcgtcgccggcggctcctcctccggcggcggcggcgagggcggcaagcccggcgccggcgagcacggcctcctccagcgccagcgccagctcgcccccgtcggcgtcatggcc

SEQ ID NO: 9 - DNA, 2238 bp, Artificial Sequence
  crtR gene
atggccaccctctccgacctcgtcatcctcctcctcggcgccctcctcgccctcggcttctacaacaaggaccgcctcctcggctcctcctcctcctccgcctccaccacctccggctcctccgccgccaccgccaacggctccaagcccacctactccaacggcaacggcaacgccttcaagggcgacccccgcgacttcgtcgcccgcatgaaggaccagaagaagcgcctcgccgtcttctacggctcccagaccggcaccgccgaggagtacgccacccgcatcgccaaggaggccaagtcccgcttcggcgtctcctccctcgtctgcgacatcgaggagtacgacttcgagaagctcgaccaggtccccgaggactgcgccatcgtcttctgcatggccacctacggcgagggcgagcccaccgacaacgccgtccagttcatcgagatgatctcccaggacgaccccgagttctccgagggctccaccctcgacggcctcaagtacgtcgtcttcggcctcggcaacaagacctacgagcagtacaacgtcgtcggccgccagctcgacgcccgcctcaccgccctcggcgccacccgcgtcggcgagcgcggcgagggcgacgacgacaagtccatggaggaggactacctcgcctggaaggacgacatgttcgccgccctcgccaccaccctctccttcgaggagggcgcctccggcgagacccccgacttcgtcgtcaccgaggtccccaaccaccccatcgagaaggtcttccagggcgagctctcctcccgcgccctcctcggctccaagggcgtccacgacgccaagaacccctacgcctcccccgtcctcgcctgccgcgagctcttcaccggcggcgaccgcaactgcatccacctcgagttcgacatcaccggctccggcatcacctaccagaccggcgaccacgtcgccgtctggccctccaaccccgacgtcgaggtcgagcgcctcctcgccgtcctcggcctcacctcccccgagaagcgccgcatgatcatccaggtcgtctccctcgaccccaccctcgccaaggtccccttccccacccccaccacctacgacgccgtcttccgccactacctcgacatctccgccgtcgcctcccgccagaccctcgccgtcctcgccaagtacgccccctccgagcaggccgccgagttcctcacccgcctcggcaccgacaagcaggcctaccacaccgaggtcgtcggcggccacctccgcctcgccgaggtcctccagctcgccgccggcaacgacatcaccgtcatgcccaccgccgagaacaccaccgtctggaacatccccttcgaccacgtcgtctccgacgtctcccgcctccagccccgcttctactccatctcctcctcccccaagctccaccccaactccatccacgtcaccgccgtcatcctcaagtacgagtcccaggccaccgaccgccaccccgcccgctgggtcttcggcctcggcaccaactacctcctcaacgtcaagcaggccgccaacaacgagaccacccccatgatctccgacggccaggacgacgtccccgagcacgtctccgcccccaagtacaccctcgagggcccccgcggctcctacaagcacgacgaccagctcttcaaggtccccatccacgtccgccgctccaccttccgcctccccacctcccccaagatccccgtcatcatgatcggccccggcaccggcgtcgcccccttccgcggcttcatccaggagcgcatcgccctcgcccgccgctccatcgccaagaacggccccgacgccctcgccgactgggcccccatctacctcttctacggctcccgcgacgagcaggacttcctctacgccgaggagtggcccgcctacgaggccgagctccagggcaagttcaagatccacgtcgccttctcccgctccggcccccgcaagcccgacggctccaagatctacgtccaggacctcctctgggaccagaaggaggtcatcaagtccgccatcgtcgagaagcgcgcctccgtctacatctgcggcgacggccgcaacatgtccaaggacgtcgagcagaagctcgccgccatgctcgccgagtccaagaacggctccgccgccgtcgagggcgccgccgaggtcaagtccctcaaggagcgctcccgcctcctcatggacgtctggtcc

SEQ ID NO: 10 - DNA, 1671 bp, Artificial Sequence
  crtS gene
atgttcatcctcgtcctcctcaccggcgccctcggcctcgccgccttctcctgggcctccatcgccttcttctccctctacctcgccccccgccgctcctccctctacaacctccagggccccaaccacaccaactacttcaccggcaacttcctcgacatcctctccgcccgcaccggcgaggagcacgccaagtaccgcgagaagtacggctccaccctccgcttcgccggcatcgccggcgcccccgtcctcaactccaccgaccccaaggtcttcaaccacgtcatgaaggaggcctacgactaccccaagcccggcatggccgcccgcgtcctccgcatcgccaccggcgacggcgtcgtcaccgccgagggcgaggcccacaagcgccaccgccgcatcatgatcccctccctctccgcccaggccgtcaagtccatggtccccatcttcctcgagaagggcatggagctcgtcgacaagatgatggaggacgccgccgagaaggacatggccgtcggcgagtccgccggcgagaagaaggccacccgcctcgagaccgagggcgtcgacgtcaaggactgggtcggccgcgccaccctcgacgtcatggccctcgccggcttcgactacaagtccgactccctccagaacaagaccaacgagctctacgtcgccttcgtcggcctcaccgacggcttcgcccccaccctcgactccttcaaggccatcatgtgggacttcgtcccctacttccgcaccatgaagcgccgccacgagatccccctcacccagggcctcgccgtctcccgccgcgtcggcatcgagctcatggagcagaagaagcaggccgtcctcggctccgcctccgaccaggccgtcgacaagaaggacgtccagggccgcgacatcctctccctcctcgtccgcgccaacatcgccgccaacctccccgagtcccagaagctctccgacgaggaggtcctcgcccagatctccaacctcctcttcgccggctacgagacctcctccaccgtcctcacctggatgttccaccgcctctccgaggacaaggccgtccaggacaagctccgcgaggagatctgccagatcgacaccgacatgcccaccctcgacgagctcaacgccctcccctacctcgaggccttcgtcaaggagtccctccgcctcgaccccccctccccctacgccaaccgcgagtgcctcaaggacgaggacttcatccccctcgccgagcccgtcatcggccgcgacggctccgtcatcaacgaggtccgcatcaccaagggcaccatggtcatgctccccctcttcaacatcaaccgctccaagttcatctacggcgaggacgccgaggagttccgccccgagcgctggctcgaggacgtcaccgactccctcaactccatcgaggccccctacggccaccaggcctccttcatctccggcccccgcgcctgcttcggctggcgcttcgccgtcgccgagatgaaggccttcctcttcgtcaccctccgccgcgtccagttcgagcccatcatctcccaccccgagtacgagcacatcaccctcatcatctcccgcccccgcatcgtcggccgcgagaaggagggctaccagatgcgcctccaggtcaagcccgtcgag

SEQ ID NO: 11 - DNA, 26 bp, Artificial Sequence
  Forward Primer-crtE gene-AgeI
accggtatggattacgcgaacatcct

SEQ ID NO: 12 - DNA, 26 bp, Artificial Sequence
  Reverse Primer-crtE gene-NcoI
ccatggtcacagagggatatcggcta

SEQ ID NO: 13 - DNA, 28 bp, Artificial Sequence
  Forward Primer-HMG1 gene-NotI
gcggccgcatggaactaactgctaatga

SEQ ID NO: 14 - DNA, 26 bp, Artificial Sequence
  Reverse Primer-HMG1 gene-XhoI
ctcgagtcacgatttgatgcaaatca

SEQ ID NO: 15 - DNA, 26 bp, Artificial Sequence
  Forward Primer-crtI gene-AgeI
accggtatgggaaaagaacaagatca

SEQ ID NO: 16 - DNA, 26 bp, Artificial Sequence
  Reverse Primer-crtI gene-NcoI
ccatggtcagaaagcaagaacaccaa

SEQ ID NO: 17 - DNA, 26 bp, Artificial Sequence
  Forward Primer-crtYB gene-AgeI
accggtatgacggctctcgcatatta

SEQ ID NO: 18 - DNA, 28 bp, Artificial Sequence
  Reverse Primer-crtYB gene-NotI
gcggccgcttactgcccttcccatccgc

SEQ ID NO: 19 - DNA, 26 bp, Artificial Sequence
  Forward Primer-crtR gene-NcoI
ccatggatggccacactctccgatct

SEQ ID NO: 20 - DNA, 33 bp, Artificial Sequence
  Reverse Primer-crtR gene-SfiI
ggcccaacaggccctacgaccagacgtccatca

SEQ ID NO: 21 - DNA, 26 bp, Artificial Sequence
  Forward Primer-crtS gene-AgeI
accggtatgttcatcttggtcttgct

SEQ ID NO: 22 - DNA, 26 bp, Artificial Sequence
  Reverse Primer-crtS gene-NcoI
ccatggtcattcgaccggcttgacct

SEQ ID NO: 23 - DNA, 25 bp, Artificial Sequence
  primer-KlPLac4
ccgcggggatcgactcataaaatag

SEQ ID NO: 24 - DNA, 82 bp, Artificial Sequence
  primer-ScTTPGK-KlPGapDH
ggactccagcttttccatttgccttcgcgcttgcctgtacggtcgttaccatactaagctttttcgaaacgcagaattttcg

SEQ ID NO: 25 - DNA, 25 bp, Artificial Sequence
  primer-KlPGapDH
agtatggtaacgaccgtacaggcaa

SEQ ID NO: 26 - DNA, 78 bp, Artificial Sequence
  primer-ScTTGap-ScPADHI
ggaatcccgatgtatgggtttggttgccagaaaagaggaagtccatattgtacactggcggaaaaaattcatttgtaa

SEQ ID NO: 27 - DNA, 26 bp, Artificial Sequence
  primer-ScPADHI
gtgtacaatatggacttcctcttttc

SEQ ID NO: 28 - DNA, 23 bp, Artificial Sequence
  primer-ScTTADHI-KlPLac4
gaaatttaggaattttaaacttg

SEQ ID NO: 29 - DNA, 78 bp, Artificial Sequence
  primer-ScTTGap-ScPGK
ggactccagcttttccatttgccttcgcgcttgcctgtacggtcgttaccatacttggcggaaaaaattcatttgtaa

SEQ ID NO: 30 - DNA, 25 bp, Artificial Sequence
  primer-ScPGK
actgtaattgcttttagttgtgtat

SEQ ID NO: 31 - DNA, 80 bp, Artificial Sequence
  primer-ScTTPGK-KlPADHI
aggtaagtatggtaacgaccgtacaggcaagcgcgaaggcaaatggaaaagctggaagctttttcgaaacgcagaatttt

SEQ ID NO: 32 - DNA, 30 bp, Artificial Sequence
  primer-KlPADHI
ccagcttttccatttgccttcgcgcttgcc

SEQ ID NO: 33 - DNA, 78 bp, Artificial Sequence
  primer-KlTTLac4-ScPGapDH
ctactattaattatttacgtattctttgaaatggcagtattgataatgataaacttatacaacatcgaagaagagtct

SEQ ID NO: 34 - DNA, 25 bp, Artificial Sequence
  primer-ScPGapDH
agtttatcattatcaatactgccat

SEQ ID NO: 35 - DNA, 81 bp, Artificial Sequence
  primer-ScTTGap-KlPGK
catatacctttgataccataaaaacaagcaaatattcttacttcaaacacacccgtggcggaaaaaattcatttgtaaact

SEQ ID NO: 36 - DNA, 25 bp, Artificial Sequence
  primer-KlPGK
cgggtgtgtttgaagtaagaatatt

SEQ ID NO: 37 - DNA, 20 bp, Artificial Sequence
  primer-crtE-UPL 1-F
cgagatgctttccctccata

SEQ ID NO: 38 - DNA, 21 bp, Artificial Sequence
  primer-crtE-UPL 1-R
ttcgctaggacacgtcagact

SEQ ID NO: 39 - DNA, 20 bp, Artificial Sequence
  primer-crtI-UPL 155-F
ccgatccttccttttacgtg

SEQ ID NO: 40 - DNA, 20 bp, Artificial Sequence
  primer-crtI-UPL 155-R
cggcacaagaatgacgatag

SEQ ID NO: 41 - DNA, 20 bp, Artificial Sequence
  primer-crtR-UPL 41-F
acgtcgtctctgacgtttcc

SEQ ID NO: 42 - DNA, 20 bp, Artificial Sequence
  primer-crtR-UPL 41-R
ttgggtgaagtttcggagaa

SEQ ID NO: 43 - DNA, 20 bp, Artificial Sequence
  primer-crtS-UPL 149-F
ggatgttcaaggtcgggata

SEQ ID NO: 44 - DNA, 21 bp, Artificial Sequence
  primer-crtS-UPL 149-R
cggacagcttttgagattcag

SEQ ID NO: 45 - DNA, 25 bp, Artificial Sequence
  primer-crtYB-UPL 34-F
cactgatcttatctttcccttatcg

SEQ ID NO: 46 - DNA, 20 bp, Artificial Sequence
  primer-crtYB-UPL 34-R
gtggtctcgataggcgtctt

SEQ ID NO: 47 - DNA, 18 bp, Artificial Sequence
  primer-tHMG-UPL 119-F
ttctgctatggcgggttc

SEQ ID NO: 48 - DNA, 21 bp, Artificial Sequence
  primer-tHMG-UPL 119-R
gctgtaaccaaattcgaagca

SEQ ID NO: 49 - DNA, 19 bp, Artificial Sequence
  primer-CrBKT-UPL 159-F
gctgctgcaactggttcac

SEQ ID NO: 50 - DNA, 21 bp, Artificial Sequence
  primer-CrBKT-UPL 159-R
gcactagcggaactagcagaa

SEQ ID NO: 51 - DNA, 21 bp, Artificial Sequence
  primer-CrChYb-UPL 48-F
ttctttcacgatggattggtc

SEQ ID NO: 52 - DNA, 22 bp, Artificial Sequence
  primer-CrChYb-UPL 48-R
tgtatggtaagttggcgatagg

SEQ ID NO: 53 - DNA, 20 bp, Artificial Sequence
  primer-CZChYb-UPL 157-F
cgcccacaaattacaccatt

SEQ ID NO: 54 - DNA, 20 bp, Artificial Sequence
  primer-CZChYb-UPL 157-R
tccgaaaaacataccccaag

SEQ ID NO: 55 - DNA, 22 bp, Artificial Sequence
  primer-HpChYb 139-F
aacgacttgttcgcaatcatta

SEQ ID NO: 56 - DNA, 18 bp, Artificial Sequence
  primer-HpChYb 139-R
cccaacacgtttggcaac

SEQ ID NO: 57 - DNA, 22 bp, Artificial Sequence
  primer-Kan-UPL 144-F
agactaaactggctgacggaat

SEQ ID NO: 58 - DNA, 23 bp, Artificial Sequence
  primer-Kan-UPL 144-R
catcaggagtacggataaaatgc

SEQ ID NO: 59 - DNA, 20 bp, Artificial Sequence
  primer-Actin-UPL 9-F
gcgtagattggaacaacgtg

SEQ ID NO: 60 - DNA, 23 bp, Artificial Sequence
  primer-Actin-UPL 9-R
agaactaccggtattgtgttgga

SEQ ID NO: 61 - DNA, 20 bp, Artificial Sequence
  primer-alg9-UPL 132-F
caatcaatggcccgtatcat

SEQ ID NO: 62 - DNA, 21 bp, Artificial Sequence
  primer-alg9-UPL 132-R
tgtctcagaagcacagtttgg

SEQ ID NO: 63 - DNA, 2292 bp, Artificial Sequence
  KlLac4 promoter
ccgcggggatcgactcataaaatagtaaccttctaatgcgtatctattgactaccaaccattagtgtggttgcagaaggcggaattttcccttcttcgaatttagcttgctttttcattttttattttccatttttcagtttttgtttgtgtcgaatttagccagttgcttctccaagatgaaaaaaacccctgcgcagtttctgtgctgcaagatcctaatcgacttttccaccccccacaaaagtaaatgttcttttgttacattcgcgtgggtagctagctccccgaatcttcaaaggacttagggactgcactacatcagagtgtgttcacctggtttgctgcctggtttgaaagaaaagagcagggaactcgcgggttcccggcgaataatcatgcgatagtcctttggccttccaagtcgcatgtagagtagacaacagacagggagggcaggaaggatctttcactgagatcctgtatcttgttgggtaagtcggatgaaaggggaatcgtatgagattggagaggatgcggaagaggtaacgccttttgttaacttgtttaattattatggggcaggcgagagggggaggaatgtatgtgtgtgaggcgggcgagacggagccatccaggccaggtagaaatagagaaagccgaatgttagacaatatggcagcgtagtagagtaggtaggtaggcaagtactgctagcaaagaggagaagggtaagctcactcttcgcattccacaccgttagtgtgtcagtttgaacaaaaaaacaatcatcataccaattgatggactgtggactggcttttggaacggcttttcggactgcgattattcgtgaggaatcaaggtaggaatttggtcatatttacggacaacagtgggtgattcccatatcgagtaggaaaacgagatcatggtatcctcagatatgttgcggaaatctgttcaccgcaaagttcagggtgctctggtgggtttcggttggtctttgctttgcttctcccttgtcttgcatgttaataatagcctagcctgtgagccgaaacttagggtaggcttagtgttggaacgtacatatctatcacgttgacttggtttaaccaggcgacctggtagccagccatacccacacacgttttttgtatcttcagtatagttgtgaaaagtgtagcggaaatttgtggtccgagcaacagcgtctttttctagtagtgcggtcggttacttggttgacattggtatttggactttgttgctacaccattcactacttgaagtcgagtgtgaagggtatgatttctagtggtgaacacctttagttacgtaatgttttcattgctgttttacttgagatttcgattgagaaaaaggtatttaatagctcgaatcaatgtgagaacagagagaagatgttcttccctaactcgaaaggtatatgaggcttgtgtttcttaggagaattattattcttttgttatgttgcgcttgtagttggaaaaggtgaagagacaaaagctggaattgtgagcggataacaagctcaacacttgaaatttaggaaagagcagaatttggcaaaaaaaataaaaaaaaaataaacacacatactcatcgagaccggtggcgcgcccctaggggccggccacgcgtccatgggcggccgcttaattaaggcctgttgggccctcgagatttatacttagataagtatgtacttacaggtatatttctatgagatactgatgtatacatgcatgataatatttaaacggttattagtgccgattgtcttgtgcgataatgacgttcctatcaaagcaatacacttaccacctattacatgggccaagaaaatattttcgaacttgtttagaatattagcacagagtatatgatgttatccgttagattatgcatgattcattcctacaactttttcgtagcataaggattaattacttggatgccaataaaaaaaaaaaacatcgagaaaatttcagcatgctcagaaacaattgcagtgtatcaaagtaaaaaaaagattttcactacatgttccttttgaagaaagaaaatcatggaacattagatttacaaaaatttaaccaccgctgattaacgattagaccgttaagcgcacaacaggttattagtacagagaaagcattctgtggtgttgccccggactttcttttgcgacataggtaaatcgaataccatcatactatcttttccaatgactccctaaagaaagactcttcttcgatgttgtata

SEQ ID NO: 64 - DNA, 1047 bp, Artificial Sequence
  ScGapDH promoter
agtttatcattatcaatactgccatttcaaagaatacgtaaataattaatagtagtgattttcctaactttatttagtcaaaaaattagccttttaattctgctgtaacccgtacatgcccaaaatagggggcgggttacacagaatatataacatcgtaggtgtctgggtgaacagtttattcctggcatccactaaatataatggagcccgctttttaagctggcatccagaaaaaaaaagaatcccagcaccaaaatattgttttcttcaccaaccatcagttcataggtccattctcttagcgcaactacagagaacaggggcacaaacaggcaaaaaacgggcacaacctcaatggagtgatgcaacctgcctggagtaaatgatgacacaaggcaattgacccacgcatgtatctatctcattttcttacaccttctattaccttctgctctctctgatttggaaaaagctgaaaaaaaaggttgaaaccagttccctgaaattattcccctacttgactaataagtatataaagacggtaggtattgattgtaattctgtaaatctatttcttaaacttcttaaattctacttttatagttagtcttttttttagttttaaaacaccaagaacttagtttcgaataaacacacataaacaaacaaaaaaaccggtggcgcgcccctaggggccggccacgcgtccatgggcggccgcttaattaaggcctgttgggccctcgaggtgaatttactttaaatcttgcatttaaataaattttctttttatagctttatgacttagtttcaatttatatactattttaatgacattttcgattcattgattgaaagctttgtgttttttcttgatgcgctattgcattgttcttgtctttttcgccacatgtaatatctgtagtagatacctgatacattgtggatgctgagtgaaattttagttaataatggaggcgctcttaataattttggggatattggcttttttttttaaagtttacaaatgaattttttccgcca

SEQ ID NO: 65 - DNA, 1239 bp, Artificial Sequence
  ScPGK promoter
actgtaattgcttttagttgtgtatttttagtgtgcaagtttctgtaaatcgattaatttttttttctttcctctttttattaaccttaatttttattttagattcctgacttcaactcaagacgcacagatattataacatctgcataataggcatttgcaagaattactcgtgagtaaggaaagagtgaggaactatcgcatacctgcatttaaagatgccgatttgggcgcgaatcctttattttggcttcaccctcatactattatcagggccagaaaaaggaagtgtttccctccttcttgaattgatgttaccctcataaagcacgtggcctcttatcgagaaagaaattaccgtcgctcgtgatttgtttgcaaaaagaacaaaactgaaaaaacccagacacgctcgacttcctgtcttcctattgattgcagcttccaatttcgtcacacaacaaggtcctagcgacggctcacaggttttgtaacaagcaatcgaaggttctggaatggcgggaaagggtttagtaccacatgctatgatgcccactgtgatctccagagcaaagttcgttcgatcgtactgttactctctctctttcaaacagaattgtccgaatcgtgtgacaacaacagcctgttctcacacactcttttcttctaaccaagggggtggtttagtttagtagaacctcgtgaaacttacatttacatatatataaacttgcataaattggtcaatgcaagaaatacatatttggtcttttctaattcgtagtttttcaagttcttagatgctttctttttctcttttttacagatcatcaaggaagtaattatctactttttacaacaaatataaaacaaaaaaaaccggtggcgcgcccctaggggccggccacgcgtccatgggcggccgcttaattaaggcctgttgggccctcgagattgaattgaattgaaatcgatagatcaatttttttcttttctctttccccatcctttacgctaaaataatagtttattttattttttgaatattttttatttatatacgtatatatagactattatttacttttaatagattattaagatttttattaaaaaaaaattcgtccctctttttaatgccttttatgcagtttttttttcccattcgatatttctatgttcgggtttcagcgtattttaagtttaataactcgaaaattctgcgtttcgaaaaagctt

SEQ ID NO: 66 - DNA, 1090 bp, Artificial Sequence
  KlGapDH promoter
agtatggtaacgaccgtacaggcaagcgcgaaggcaaatggaaaagctggagtccggaagataatcatttcatcttcttttgttagaacagaacagtggatgtccctcatctcggtaacgtattgtccatgccctagaactctctgtccctaaaaagaggacaaaaacccaatggtttccccagcttccagtggagccaccgatcccactggaaaccactggacaggaagagaaaatcacggacttcctctattgaaggataattcaacactttcaccagatcccaaatgtcccgcccctattcccgtgttccatcacgtaccataacttaccatttcatcacgttctctatggcacactggtactgcttcgactgctttgcttcatcttctctatgggccaatgagctaatgagcacaatgtgctgcgaaataaagggatatctaatttatattattacattataatatgtactagtgtggttattggtaattgtacttaattttgatatataaagggtggatctttttcattttgaatcagaattggaattgcaacttgtctcttgtcactattacttaatagtaattatatttcttattaaccttttttttaagtcaaaacaccaaggacaagaactactcttcaaaggtatttcaagttatcatacgtctcacacacgcttcacagtttcaagtaaaaaaaaagaatattacacaaccggtggcgcgcccctaggggccggccacgcgtccatgggcggccgcttaattaaggcctgttgggccctcgaggtgaatttactttaaatcttgcatttaaataaattttctttttatagctttatgacttagtttcaatttatatactattttaatgacattttcgattcattgattgaaagctttgtgttttttcttgatgcgctattgcattgttcttgtctttttcgccacatgtaatatctgtagtagatacctgatacattgtggatgctgagtgaaattttagttaataatggaggcgctcttaataattttggggatattggcttttttttttaaagtttacaaatgaattttttccgcca

SEQ ID NO: 67 - DNA, 1236 bp, Artificial Sequence
  KlPGK promoter
cgggtgtgtttgaagtaagaatatttgcttgtttttatggtatcaaaggtatatgttgtagaagacaatttccggtaatccaattgtctgtctgctcagtttagcacatgtatagtacgttgcacatagtctacaatattcagcattcagcattcagtatacagcatatggctaaatgatcacaaatgtgattgatgatttgacacgactagaaaagagaacgaaaaagggaaattccatgtcacgtgcgttggcacgtgacatggaatatcgaagaaagaaaaaaaaaacgatctcgtcctagtggaagcccagagtctggtccccccggagtcttcccaaaacaagaagctgacacatgttgacacagaacaccccacagcaaatgcaccacgctacgtagatcaggaagcttaactctagcgacctgtcgctcgccccacagaacctcacccgagaaccacacattacacgccgccagctcccactatactcatcttgcttcccttaagcgttctcacgattcgttcgctgcccttcttcaagagtcttctgattctaattctcattcgaaatcctctacagttaatgaattgcttgacatgacattcattgtctcatggttttggctttttggcttttgtcttttaaagctatatcaactttacatataaatatacgtcaaaaggggattcattaattagaaaattctctttttcaatagttgctattcattatcaatctattcaactcaattggttattattttcatctttttgtcatcctaaaccatcaacaatatttaaatatatctgttgctacattaagagttacttcagaaataacaaaaaaatcgatcaagaattaataaaaaaaccggtggcgcgcccctaggggccggccacgcgtccatgggcggccgcttaattaaggcctgttgggccctcgagattgaattgaattgaaatcgatagatcaatttttttcttttctctttccccatcctttacgctaaaataatagtttattttattttttgaatattttttatttatatacgtatatatagactattatttacttttaatagattattaagatttttattaaaaaaaaattcgtccctctttttaatgccttttatgcagtttttttttcccattcgatatttctatgttcgggtttcagcgtattttaagtttaataactcgaaaattctgcgtttcgaaaaagctt

SEQ ID NO: 68 - DNA, 1246 bp, Artificial Sequence
  KlADHI promoter
ccagcttttccatttgccttcgcgcttgcctgtacggtcgttaccatacttacctttcttgcttcttctcaaaatggaatccaggtttttagcttcgtgtttcttttttttttttaccatttttcaaatttcagtcttccattttcagcttcttgtttttttttttttttttttttttcatttcagtttttacagcttccagtctccctctttccttcgatttccatcttcttgtttctgtagccatcttcctatcacgtgcaagggaagaaagtgggggcccagcaccttcttttttgttctttggtgggggctcgttttagtttttacgtgcgtaattgggaatcttccgaggtagtatgacatgtccggtggtgacctgatactttctgtttctccgagtaggacagaagaggaaaaaaaaatagcgtgtgatgttcttctattctagtagtgtattgatctattcacaatcagatcacaatcatatgagcagatgatgtattttgggttgcttttcaccaacccaagtattcgattgatctttatatactgcggttatttctaggtcttaaacggttaacacctgttgcagggtggtatgtatttttctcaaagtgtgctattttcacaccagctagaaatcagctgtcttacttgtatacaattagaccagccatttggtcttctggaatatgtatataaacacccggtcgattctgacaatccatccacttttgtagtaggtctctctatatccatttgtacaatgttgtttctgttttgccctacatcatcatcaagcaaaaacaatagtttcaattgaaacataaacaagctttaaacacacaaactctatactaaaaaaagataaaaccggtggcgcgcccctaggggccggccacgcgtccatgggcggccgcttaattaaggcctgttgggccctcgaggtgaatttactttaaatcttgcatttaaataaattttctttttatagctttatgacttagtttcaatttatatactattttaatgacattttcgattcattgattgaaagctttgtgttttttcttgatgcgctattgcattgttcttgtctttttcgccacatgtaatatctgtagtagatacctgatacattgtggatgctgagtgaaattttagttaataatggaggcgctcttaataattttggggatattggcttttttttttaaagtttacaaatgaattttttccgcca

SEQ ID NO: 69 - DNA, 2068 bp, Artificial Sequence
  ScADHI promoter
gtgtacaatatggacttcctcttttctggcaaccaaacccatacatcgggattcctataataccttcgttggtctccctaacatgtaggtggcggaggggagatatacaatagaacagataccagacaagacataatgggctaaacaagactacaccaattacactgcctcattgatggtggtacataacgaactaatactgtagccctagacttgatagccatcatcatatcgaagtttcactaccctttttccatttgccatctattgaagtaataataggcgcatgcaacttcttttctttttttttcttttctctctcccccgttgttgtctcaccatatccgcaatgacaaaaaaatgatggaagacactaaaggaaaaaattaacgacaaagacagcaccaacagatgtcgttgttccagagctgatgaggggtatctcgaagcacacgaaactttttccttccttcattcacgcacactactctctaatgagcaacggtatacggccttccttccagttacttgaatttgaaataaaaaaaagtttgctgtcttgctatcaagtataaatagacctgcaattattaatcttttgtttcctcgtcattgttctcgttccctttcttccttgtttctttttctgcacaatatttcaagctataccaagcatacaatcaagcaattccagatctaaaaaaaccggtggcgcgcccctaggggccggccacgcgtccatgggcggccgcttaattaaggcctgttgggccctcgagcccggggggggctcgatcccctcgcgagttggttcagctgctgcctgaggctggacgacctcgcggagttctaccggcagtgcaaatccgtcggcatccaggaaaccagcagcggctatccgcgcatccatgcccccgaactgcaggagtggggaggcacgatggccgctttggtcgatctagattacgtggaagaaaggtagtaaaagtagtagtataagtagtaaaaagaggtaaaaagagaaaaccggctacatactagagaagcacgtacacaaaaactcataggcacttcatcatacgacagtttcttgatgcattataatagtgtattagatattttcagaaatatgcatagaacctcctcttgcctttactttttatacatagaacattggcagatttacttacactactttgtttctacgccatttcttttgttttcaacacttagacaagttgttgagaaccggactactaaaaagcaatgttcccactgaaaatcatgtacctgcagcataataaccccctaattctgcatcgatccagtatgtttttttttctctactcatttttacctgaagatagagcttctaaaacaaaaaaaatcagtgattacatgcatattgtgtgttctagtaaccaaaggaaaggaacagatagataaaattccgagactgtcaaattaggtttttttctttttttttggcgggagtcagtgggccgaaatatgttcttggcctagaacttaatctggtttgatcatgccaatacttgcctgagtgcccgactttttgcccaccctcttgccttctgtcatccttcaaaacccacctgttttccagccgtatcttcgctcgcatctacacatactgtgccatatcttgtgtgtagccggacgtgactatgaccaaaaacaaacaaggagaactgttcgccgatttgtaacactcctgcatccatccaagtgggtatgcgctatgcaatgttaagctaggtcaggtcagaccaggtccaaggacagcaacttgactgtatgcaacctttaccatctttgcacagaacatacttgtagctagctagttacacttatggaccgaaaaggcaccccaccatgtctgtccggctttagagtacggccgcagaccgctgatttgccttgccaagcagtagtcacaatgcatcgcatgagcacacgggcacgggcacgggcacaggaaccattggcaaaaataccagatacactataccgacgtatatcaagcccaagtttaaaattcctaaatttc

SEQ ID NO: 70 - DNA, 28 bp, Artificial Sequence
  KlPLac4-3 SalI-F
taggtcgacccgcggggatcgactcata

SEQ ID NO: 71 - DNA, 92 bp, Artificial Sequence
  KlPLac4-3-R
aagcggccgcccatggacgcgtggccggcccctaggggcgcgccaccggtctcgatgagtatgtgtgtttattttttttttattttttttgc

SEQ ID NO: 72 - DNA, 93 bp, Artificial Sequence
  KlTTLac4-F
gccacgcgtccatgggcggccgcttaattaaggcctgttgggccctcgagatttatacttagataagtatgtacttacaggtatatttctatg

SEQ ID NO: 73 - DNA, 46 bp, Artificial Sequence
  KlTTLac4-EcoRI-R
taggaattcctactattaattatttacgtattctttgaaatggcag

SEQ ID NO: 74 - DNA, 46 bp, Artificial Sequence
  ScPGapDH-SalI-F
taggtcgacagtttatcattatcaatactgccatttcaaagaatac

SEQ ID NO: 75 - DNA, 90 bp, Artificial Sequence
  ScPGapDH-R
aagcggccgcccatggacgcgtggccggcccctaggggcgcgccaccggtttttttgtttgtttatgtgtgtttattcgaaactaagttc

SEQ ID NO: 76 - DNA, 104 bp, Artificial Sequence
  ScTTGap-F
gccacgcgtccatgggcggccgcttaattaaggcctgttgggccctcgaggtgaatttactttaaatcttgcatttaaataaattttctttttatagctttatg

SEQ ID NO: 77 - DNA, 30 bp, Artificial Sequence
  ScTTGap-EcoRI-R
taggaattcggactccagcttttccatttg

SEQ ID NO: 78 - DNA, 35 bp, Artificial Sequence
  ScPADHI-SalI-F
taggtcgacgtgtacaatatggacttcctcttttc

SEQ ID NO: 79 - DNA, 82 bp, Artificial Sequence
  ScPADHI -R
aagcggccgcccatggacgcgtggccggcccctaggggcgcgccaccggtttttttagatctggaattgcttgattgtatgc

SEQ ID NO: 80 - DNA, 75 bp, Artificial Sequence
  ScTTADHI_KlPLac4 -5 End-F
gccacgcgtccatgggcggccgcttaattaaggcctgttgggccctcgagcccggggggggctcgatcccctcgc

SEQ ID NO: 81 - DNA, 44 bp, Artificial Sequence
  ScTTADHI_KlPLac4-5 End_EcoRI-R
taggaattcgaaatttaggaattttaaacttgggcttgatatac

SEQ ID NO: 82 - DNA, 44 bp, Artificial Sequence
  ScPGK-SalI-F
taggtcgacactgtaattgcttttagttgtgtatttttagtgtg

SEQ ID NO: 83 - DNA, 100 bp, Artificial Sequence
  ScPGK-R
aagcggccgcccatggacgcgtggccggcccctaggggcgcgccaccggttttttttgttttatatttgttgtaaaaagtagataattacttccttgatg

SEQ ID NO: 84 - DNA, 94 bp, Artificial Sequence
  ScTTPGK-F
gccacgcgtccatgggcggccgcttaattaaggcctgttgggccctcgagattgaattgaattgaaatcgatagatcaatttttttcttttctc

SEQ ID NO: 85 - DNA, 46 bp, Artificial Sequence
  ScTTPGK-EcoRI-R
taggaattccatatacctttgataccataaaaacaagcaaatattc

SEQ ID NO: 86 - DNA, 30 bp, Artificial Sequence
  KlPGapDH-SalI-F
taggtcgacagtatggtaacgaccgtacag

SEQ ID NO: 87 - DNA, 88 bp, Artificial Sequence
  KlPGapDH-R
aagcggccgcccatggacgcgtggccggcccctaggggcgcgccaccggttgtgtaatattctttttttttacttgaaactgtgaagc

SEQ ID NO: 88 - DNA, 104 bp, Artificial Sequence; identical to SEQ ID NO: 76
  ScTTGap-F

SEQ ID NO: 89 - DNA, 49 bp, Artificial Sequence
  ScTTGap-EcoRI-R
taggaattctggcggaaaaaattcatttgtaaactttaaaaaaaaaagc

SEQ ID NO: 90 - DNA, 36 bp, Artificial Sequence
  KlPGK-SalI-F
taggtcgaccgggtgtgtttgaagtaagaatatttg

SEQ ID NO: 91 - DNA, 98 bp, Artificial Sequence
  KlPGK -R
aagcggccgcccatggacgcgtggccggcccctaggggcgcgccaccggtttttttattaattcttgatcgatttttttgttatttctgaagtaactc

SEQ ID NO: 92 - DNA, 94 bp, Artificial Sequence; identical to SEQ ID NO: 84
  ScTTPGK -F

SEQ ID NO: 93 - DNA, 36 bp, Artificial Sequence
  ScTTPGK-EcoRI-R
taggaattcaagctttttcgaaacgcagaattttcg

SEQ ID NO: 94 - DNA, 30 bp, Artificial Sequence
  KlPADHI-SalI-F
taggtcgacccagcttttccatttgccttc

SEQ ID NO: 95 - DNA, 91 bp, Artificial Sequence
  KlPADHI -R
aagcggccgcccatggacgcgtggccggcccctaggggcgcgccaccggttttatctttttttagtatagagtttgtgtgtttaaagcttg

SEQ ID NO: 96 - DNA, 104 bp, Artificial Sequence; identical to SEQ ID NO: 76
  ScTTGap-F

SEQ ID NO: 97 - DNA, 28 bp, Artificial Sequence
  ScTTGap-EcoRI-R
taggaattcggaatcccgatgtatgggt

SEQ ID NO: 98 - DNA, 26 bp, Artificial Sequence
  Forward Primer-kan gene-AgeI
accggtatgggtaaggaaaagactca

SEQ ID NO: 99 - DNA, 26 bp, Artificial Sequence
  Reverse Primer-kan gene-NcoI
ccatggttagaaaaactcatcgagca

SEQ ID NO: 100 - protein, 61 aa, Artificial Sequence
  catalytic domain 1
  VARIANT 2,3,4,5,6,7,8,10,11,12,13,15,18,21,24,25,30,33,37,38,41,42,43,44,47,54,57: Xaa is any amino acid
HXXXXXXXPXXXXAXTLXLVXGGXXGMEMXARXAHKXXWHXXXXGWXLHKSHHXPRXGPFE

SEQ ID NO: 101 - protein, 76 aa, Artificial Sequence
  catalytic domain 2
  VARIANT 3,4,7,8,11,12,14,15,16,18,19,30,32,33,37,44,48,53,54,56,60,61,62,65,66,69,70,72,75: Xaa is any amino acid
PAXXLCXXGFXXPXXXGXXCFGAGLGITLXGXXYMFXHDGLVHXRFPXGPIAXXPXMKRXXXAHXXHHXXKXGGXP

SEQ ID NO: 102 - protein, 61 aa, Artificial Sequence
  catalytic domain 1-Chlamydomonas reinhardtii
HFAEDGDLPVDEMAATLLLVFGGMFGMEMYARFAHKVLWHDFEPGWALHKSHHEPRTGPFE

SEQ ID NO: 103 - protein, 61 aa, Artificial Sequence
  catalytic domain 1-Chromochloris zofingiensis
HMPSESPFPWLDMAGTLALVIGGVFGMEMWARYAHKALWHDFQPGWALHKSHHEPRIGPFE

SEQ ID NO: 104 - protein, 61 aa, Artificial Sequence
  catalytic domain 1-Haematococcus pluvialis
HMTVGGAVPWGEVAGTLLLVVGGALGMEMYARYAHKAIWHESPLGWLLHKSHHTPRTGPFE

SEQ ID NO: 105 - protein, 76 aa, Artificial Sequence
  catalytic domain 2-Chlamydomonas reinhardtii
PAMALCAYGFFTPHVIGGVCFGAGLGITLFGIAYMFFHDGLVHRRFPVGPIANLPYMKRIMVAHQIHHTNKFGGVP

SEQ ID NO: 106 - protein, 76 aa, Artificial Sequence
  catalytic domain 2-Chromochloris zofingiensis
PAFSLCLYGFLTPNLVGSLCFGAGLGITLFGIMYMFIHDGLVHKRFPVGPIAQMPAMKRVAIAHKLHHSEKYGGVP

SEQ ID NO: 107 - protein, 76 aa, Artificial Sequence
  catalytic domain 2-Haematococcus pluvialis
PAMLLCTFGFWLPNVLGAACFGAGLGITLYGMAYMFVHDGLVHRRFPTGPIAGLPYMKRLTVAHQLHHSGKYGGAP

SEQ ID NO: 108 - DNA, 26 bp, Artificial Sequence
  synthetic
gtgtacaatatggacttcctcttttc

SEQ ID NO: 109 - DNA, 26 bp, Artificial Sequence
  synthetic
gaaaagaggaagtccatattgtacac

SEQ ID NO: 110 - protein, 30 aa, Artificial Sequence
  synthetic
  VARIANT 2,3,4,5,8,9,10,11,12,13,17,18,19,22,23,24,26,28,29: Xaa is any amino acid
PXXXXDYXXXXXXCCEXXXGYXXXPXGXXG

SEQ ID NO: 111 - protein, 39 aa, Artificial Sequence
  synthetic
  VARIANT 2,3,5,8,13,14,20,21,22,23,26,28,29,30,31,32,34,38: Xaa is any amino acid
PXXTXEGXLVASXXRGCKAXXXXGGXTXXXXXDXMTRXP

SEQ ID NO: 112 - protein, 20 aa, Artificial Sequence
  synthetic
  VARIANT 2,3,4,5,6,9,10,11: Xaa is any amino acid
GXXXXXRFXXXTGDAMGMNM

SEQ ID NO: 113 - protein, 17 aa, Artificial Sequence
  synthetic
  VARIANT 2,9,10,12: Xaa is any amino acid
CXDKKPAAXXWXEGRGK

SEQ ID NO: 114 - protein, 31 aa, Artificial Sequence
  synthetic
  VARIANT 6,8,10,11,12,14,15,16,18,22,30: Xaa is any amino acid
GGFNAXAXNXXXAXXXAXGQDXAQNVESSXC

SEQ ID NO: 115 - protein, 36 aa, Artificial Sequence
  synthetic
  VARIANT 3,4,9,14,16,17,19,21,23,28,30,31,32,33,34: Xaa is any amino acid
MPXXEVGTXGGGTXLXXQXAXLXLLGVXGXXXXXPG

SEQ ID NO: 116 - protein, 20 aa, Artificial Sequence
  synthetic
  VARIANT 2,3,6,7,9,11,12,16,18,19: Xaa is any amino acid
LXXDDXXDXSXXRRGXPXXH

SEQ ID NO: 117 - protein, 6 aa, Artificial Sequence
  synthetic
  VARIANT 3,4: Xaa is any amino acid
FQXXDD

SEQ ID NO: 118 - protein, 18 aa, Artificial Sequence
  synthetic
  VARIANT 2,3,5,7,8,9,10,11,12,13,14,16,17: Xaa is any amino acid
YXXWXDXXXXXXXXWXXN

SEQ ID NO: 119 - protein, 8 aa, Artificial Sequence
  synthetic
  VARIANT 2,3,4,5,6: Xaa is any amino acid
PXXXXXFF

SEQ ID NO: 120 - protein, 12 aa, Artificial Sequence
  synthetic
  VARIANT 2,3,6,7,9,10,11: Xaa is any amino acid
YXXCRXXDXXXD

SEQ ID NO: 121 - protein, 22 aa, Artificial Sequence
  synthetic
  VARIANT 2,3,4,8,10,11,12,13,14,15,16,17,18,19,20,21: Xaa is any amino acid
YXXXVAGXVXXXXXXXXXXXXP

SEQ ID NO: 122 - protein, 48 aa, Artificial Sequence
  synthetic
  VARIANT 2,7,8,9,11,12,14,15,16,18,19,20,21,23,25,26,27,28,29,32,33,34,35,36,37,39,42,45,47: Xaa is any amino acid
GXGIGGXXXAXXLXXXGXXXXVXEXXXXXGGXXXXXXRXGYXFDXGXS

SEQ ID NO: 123 - protein, 14 aa, Artificial Sequence
  synthetic
  VARIANT 2,3,4,5,7,8,9,10,11,12,13: Xaa is any amino acid
RXXXXPXXXXXXXK

SEQ ID NO: 124 - protein, 29 aa, Artificial Sequence
  synthetic
  VARIANT 2,3,5,6,7,8,9,10,11,12,13,14,15,17,18,19,20,21,22,24,25,26,27,28: Xaa is any amino acid
GXXTXXXXXXXXXXXLXXXXXXQXXXXXE

SEQ ID NO: 125 - protein, 22 aa, Artificial Sequence
  synthetic
  VARIANT 2,3,7,9,11,12,14,15,16,17,18,19,20,21: Xaa is any amino acid
FXXGPRXCXGXXFXXXXXXXXL

SEQ ID NO: 126 - protein, 19 aa, Artificial Sequence
  synthetic
  VARIANT 2,11,12,14,15,16,17,18: Xaa is any amino acid
FXGSQTGTAEXXAXXXXXE

SEQ ID NO: 127 - protein, 33 aa, Artificial Sequence
  synthetic
  VARIANT 2,3,4,5,6,7,10,11,12,13,14,15,16,17,18,20,21: Xaa is any amino acid
EXXXXXXLDXXXXXXXXXFXXATYGEGEPTDNA

SEQ ID NO: 128 - protein, 41 aa, Artificial Sequence
  synthetic
  VARIANT 2,3,9,13,14,16,17,18,19,20,21,24,25,26,27,30,31,33,35,36,38: Xaa is any amino acid
YXXFGLGNXTYEXXNXXXXXXDAXXXXLGXXRXGXXGXGDD

SEQ ID NO: 129 - protein, 8 aa, Artificial Sequence
  synthetic
  VARIANT 4,6: Xaa is any amino acid
EEDXLXWK

SEQ ID NO: 130 - protein, 14 aa, Artificial Sequence
  synthetic
  VARIANT 3,4,5,6,7,8,9,10,11: Xaa is any amino acid
NPXXXXXXXXXELF

SEQ ID NO: 131 - protein, 21 aa, Artificial Sequence
  synthetic
  VARIANT 2,4,6,8,9,11,12,14,15,16,19: Xaa is any amino acid
RXCXHXEXXIXXSXXXYQXGD

SEQ ID NO: 132 - protein, 37 aa, Artificial Sequence
  synthetic
  VARIANT 2,4,5,6,11,12,13,14,16,18,19,20,21,22,23,24,28,29,30,31,32,34,35: Xaa is any amino acid
KXPXXXPTTYXXXXRXYXXXXXXXSRQXXXXXAXXAP

SEQ ID NO: 133 - protein, 22 aa, Artificial Sequence
  synthetic
  VARIANT 3,4,5,6,7,8,9,10,11,12,13,16: Xaa is any amino acid
PFXXXXXXXXXXXPRXYSISSS

SEQ ID NO: 134 - protein, 21 aa, Artificial Sequence
  synthetic
  VARIANT 2,5,16,18,19,20: Xaa is any amino acid
PXIMXGPGTGVAPFRXFXXXR

SEQ ID NO: 135 - protein, 15 aa, Artificial Sequence
  synthetic
  VARIANT 3,9,10,13: Xaa is any amino acid
FLXTGLFIXXHDXMH

SEQ ID NO: 136 - protein, 22 aa, Artificial Sequence
  synthetic
  VARIANT 4,5,6,7,8,9,10,11,12,13,15,16,17,19,20,21: Xaa is any amino acid
DPDXXXXXXXXXXWXXXFXXXY

SEQ ID NO: 137 - protein, 22 aa, Artificial Sequence
  synthetic
  VARIANT 2,3,4,5,6,7,8,10,11,12,15,16,19,20: Xaa is any amino acid
FXXXXXXXSXXXLFXXGTXXPH

SEQ ID NO: 138 - protein, 26 aa, Artificial Sequence
  synthetic
  VARIANT 3,4,7,9,10,12,16,17,19,20,23,24: Xaa is any amino acid
SFXXCYXFXXHXEHHXXPXXPWXXLP

SEQ ID NO: 139 - DNA, 25 bp, Artificial Sequence
  synthetic
agtatggtaacgaccgtacaggcaa

SEQ ID NO: 140 - DNA, 25 bp, Artificial Sequence
  synthetic
ttgcctgtacggtcgttaccatact